European Patent Application EP 4 112 050 A1, published January 4, 2023. Title: USE OF NUCLEOSIDE COMPOUND IN TREATMENT OF CORONAVIRUS INFECTIOUS DISEASES. Applicant: HENAN GENUNIE BIOTECH CO., LTD. The sequence listing filed with the application follows.

SEQUENCE LISTING (2 sequences)

SEQ ID NO: 1 - DNA, 21 bp, Artificial Sequence
  RBD-qF1
caatggtttaacaggcacagg

SEQ ID NO: 2 - DNA, 21 bp, Artificial Sequence
  RBD-qR1
ctcaagtgtctgtggatcacg